European Patent Specification EP 3 625 339 B1, published September 3, 2025. Title: Modifications to Lysine Decarboxylase Enzymes. Applicant: CATHAY R&D CENTER CO., LTD. CATHAY INDUSTRIAL BIOTECH LTD. The sequence listing filed with the application follows.

SEQUENCE LISTING (51 sequences)

SEQ ID NO: 1 - DNA, 2148 bp, Escherichia coli
atgaacgttattgcaatattgaatcacatgggggtttattttaaagaagaacccatccgtgaacttcatcgcgcgcttgaacgtctgaacttccagattgtttacccgaacgaccgtgacgacttattaaaactgatcgaaaacaatgcgcgtctgtgcggcgttatttttgactgggataaatataatctcgagctgtgcgaagaaattagcaaaatgaacgagaacctgccgttgtacgcgttcgctaatacgtattccactctcgatgtaagcctgaatgacctgcgtttacagattagcttctttgaatatgcgctgggtgctgctgaagatattgctaataagatcaagcagaccactgacgaatatatcaacactattctgcctccgctgactaaagcactgtttaaatatgttcgtgaaggtaaatatactttctgtactcctggtcacatgggcggtactgcattccagaaaagcccggtaggtagcctgttctatgatttctttggtccgaataccatgaaatctgatatttccatttcagtatctgaactgggttctctgctggatcacagtggtccacacaaagaagcagaacagtatatcgctcgcgtctttaacgcagaccgcagctacatggtgaccaacggtacttccactgcgaacaaaattgttggtatgtactctgctccagcaggcagcaccattctgattgaccgtaactgccacaaatcgctgacccacctgatgatgatgagcgatgttacgccaatctatttccgcccgacccgtaacgcttacggtattcttggtggtatcccacagagtgaattccagcacgctaccattgctaagcgcgtgaaagaaacaccaaacgcaacctggccggtacatgctgtaattaccaactctacctatgatggtctgctgtacaacaccgacttcatcaagaaaacactggatgtgaaatccatccactttgactccgcgtgggtgccttacaccaacttctcaccgatttacgaaggtaaatgcggtatgagcggtggccgtgtagaagggaaagtgatttacgaaacccagtccactcacaaactgctggcggcgttctctcaggcttccatgatccacgttaaaggtgacgtaaacgaagaaacctttaacgaagcctacatgatgcacaccaccacttctccgcactacggtatcgtggcgtccactgaaaccgctgcggcgatgatgaaaggcaatgcaggtaagcgtctgatcaacggttctattgaacgtgcgatcaaattccgtaaagagatcaaacgtctgagaacggaatctgatggctggttctttgatgtatggcagccggatcatatcgatacgactgaatgctggccgctgcgttctgacagcacctggcacggcttcaaaaacatcgataacgagcacatgtatcttgacccgatcaaagtcaccctgctgactccggggatggaaaaagacggcaccatgagcgactttggtattccggccagcatcgtggcgaaatacctcgacgaacatggcatcgttgttgagaaaaccggtccgtataacctgctgttcctgttcagcatcggtatcgataagaccaaagcactgagcctgctgcgtgctctgactgactttaaacgtgcgttcgacctgaacctgcgtgtgaaaaacatgctgccgtctctgtatcgtgaagatcctgaattctatgaaaacatgcgtattcaggaactggctcagaatatccacaaactgattgttcaccacaatctgccggatctgatgtatcgcgcatttgaagtgctgccgacgatggtaatgactccgtatgctgcattccagaaagagctgcacggtatgaccgaagaagtttacctcgacgaaatggtaggtcgtattaacgccaatatgatccttccgtacccgccgggagttcctctggtaatgccgggtgaaatgatcaccgaagaaagccgtccggttctggagttcctgcagatgctgtgtgaaatcggcgctcactatccgggctttgaaaccgatattcacggtgcataccgtcaggctgatggccgctataccgttaaggtattgaaagaagaaagcaaaaaataa

SEQ ID NO: 2 - protein, 715 aa, Escherichia coli
MNVIAILNHMGVYFKEEPIRELHRALERLNFQIVYPNDRDDLLKLIENNARLCGVIFDWDKYNLELCEEISKMNENLPLYAFANTYSTLDVSLNDLRLQISFFEYALGAAEDIANKIKQTTDEYINTILPPLTKALFKYVREGKYTFCTPGHMGGTAFQKSPVGSLFYDFFGPNTMKSDISISVSELGSLLDHSGPHKEAEQYIARVFNADRSYMVTNGTSTANKIVGMYSAPAGSTILIDRNCHKSLTHLMMMSDVTPIYFRPTRNAYGILGGIPQSEFQHATIAKRVKETPNATWPVHAVITNSTYDGLLYNTDFIKKTLDVKSIHFDSAWVPYTNFSPIYEGKCGMSGGRVEGKVIYETQSTHKLLAAFSQASMIHVKGDVNEETFNEAYMMHTTTSPHYGIVASTETAAAMMKGNAGKRLINGSIERAIKFRKEIKRLRTESDGWFFDVWQPDHIDTTECWPLRSDSTWHGFKNIDNEHMYLDPIKVTLLTPGMEKDGTMSDFGIPASIVAKYLDEHGIVVEKTGPYNLLFLFSIGIDKTKALSLLRALTDFKRAFDLNLRVKNMLPSLYREDPEFYENMRIQELAQNIHKLIVHHNLPDLMYRAFEVLPTMVMTPYAAFQKELHGMTEEVYLDEMVGRINANMILPYPPGVPLVMPGEMITEESRPVLEFLQMLCEIGAHYPGFETDIHGAYRQADGRYTVKVLKEESKK

SEQ ID NO: 3 - protein, 715 aa, Klebsiella
MNVIAIMNHMGVYFKEEPIRELHRALERLDFRIVYPNDRDDLLKLIENNSRLCGVIFDWDKYNLELCEEISKMNEYMPLYAFANTYSTLDVSLNDLRMQVRFFEYALGAAEDIANKIKQNTDEYIDTILPPLTKALFKYVREGKYTFCTPGHMGGTAFQKSPVGSIFYDFFGPNTMKSDISISVSELGSLLDHSGPHKEAEEYIARVFNAERSYMVTNGTSTANKIVGMYSAPAGSTVLIDRNCHKSLTHLMMMSDITPIYFRPTRNAYGILGGIPQSEFQHATIAKRVKETPNATWPVHAVITNSTYDGLLYNTDFIKKTLDVKSIHFDSAWVPYTNFSPIYEGKCGMSGGRVEGKVIYETQSTHKLLAAFSQASMIHVKGDVNEETFNEAYMMHTTTSPHYGIVASTETAAAMMKGNAGKRLIDGSIERSIKFRKEIKRLKGESDGWFFDVWQPEHIDGPECWPLRSDSAWHGFKNIDNEHMYLDPIKVTLLTPGMKKDGTMDDFGIPASIVAKYLDEHGIVVEKTGPYNLLFLFSIGIDKTKALSLLRALTDFKRAFDLNLRVKNMLPSLYREDPEFYENMRIQDLAQNIHKLIEHHNLPDLMFRAFEVLPSMVMTPYAAFQKELHGQTEEVYLEEMVGRVNANMILPYPPGVPLVMPGEMITEESRPVLEFLQMLCEIGAHYPGFETDIHGAYRQADGRYTVKVLKEENNK

SEQ ID NO: 4 - protein, 715 aa, Enterobacteriaceae
MNVIAIMNHMGVYFKEEPIRELHRALERLDFRIVYPNDRDDLLKLIENNSRLCGVIFDWDKYNLELCEEISKMNEYMPLYAFANTYSTLDVSLNDLRMQVRFFEYALGAAEDIANKIKQNTDEYIDTILPPLTKALFKYVREGKYTFCTPGHMGGTAFQKSPVGSIFYDFFGSNTMKSDISISVSELGSLLDHSGPHKEAEEYIARVFNAERSYMVTNGTSTANKIVGMYSAPAGSTVLIDRNCHKSLTHLMMMSDITPIYFRPTRNAYGILGGIPQSEFQHATIAKRVKETPNATWPVHAVITNSTYDGLLYNTDFIKKTLDVKSIHFDSAWVPYTNFSPIYEGKCGMSGGRVEGKVIYETQSTHKLLAAFSQASMIHVKGDVNEETFNEAYMMHTTTSPHYGIVASTETAAAMMKGNAGKRLIDGSIERSIKFRKEIKRLKGESDGWFFDVWQPEHIDGPECWPLRSDSAWHGFKNIDNEHMYLDPIKVTLLTPGMKKDGTMDDFGIPASIVAKYLDEHGIVVEKTGPYNLLFLFSIGIDKTKALSLLRALTDFKRAFDLNLRVKNMLPSLYREDPEFYENMRIQDLAQNIHKLIEHHNLPDLMFRAFEVLPSMVMTPYAAFQKELHGQTEEVYLEEMVGRVNANMILPYPPGVPLVMPGEMITEESRPVLEFLQMLCEIGAHYPGFETDIHGAYRQADGRYTVKVLKEENNK

SEQ ID NO: 5 - protein, 714 aa, Salmonella enterica
MNVIAIMNHMGVYFKEEPIRELHRALEGLNFRIVYPNDREDLLKLIENNSRLCGVIFDWDKYNLELCEEISKLNEYMPLYAFANSYSTLDVSLNDLRMQVRFFEYALGAATDIAAKIRQNTDEYIDNILPPLTKALFKYVREGKYTFCTPGHMGGTAFQKSPVGSIFYDFFGPNTMKSDISISVSELGSLLDHSGPHKEAEEYIARVFNAERSYMVTNGTSTANKIVGMYSAPAGSTVLIDRNCHKSLTHLMMMSDITPIYFRPTRNAYGILGGIPQSEFQHATIAKRVKETPNATWPVHAVITNSTYDGLLYNTDYIKKTLDVKSIHFDSAWVPYTNFSPIYQGKCGMSGDRVEGKIIYETQSTHKLLAAFSQASMIHVKGDINEETFNEAYMMHTTTSPHYGIVASTETAAAMMKGNAGKRLINGSIERAIKFRKEIKRLKSESDGWFFDVWQPEHIDGAECWPLRSDSAWHGFKNIDNEHMYLDPIKVTILTPGMKKDGTMDEFGIPASLVAKYLDERGIIVEKTGPYNLLFLFSIGIDKTKALSLLRALTEFKRAFDLNLRVKNILPALYREAPEFYENMRIQELAQNIHKLVEHHNLPDLMYRAFEVLPKMVMTPYTAFQKELHGETEEVYLEEMVGRVNANMILPYPPGVPLVMPGEMITEESRPVLEFLQMLCEIGAHYPGFETDIHGAYRQADGRYTVKVLKENTK

SEQ ID NO: 6 - DNA, 52 bp, Artificial Sequence
  Primer cadA-F
ggcgagctcacacaggaaacagaccatgaacgttattgcaatattgaatcac

SEQ ID NO: 7 - DNA, 28 bp, Artificial Sequence
  Primer cadA-R
ggctctagaccacttcccttgtacgagc

SEQ ID NO: 8 - DNA, 44 bp, Artificial Sequence
  Primer cadA-F2
atttcacacaggaaacagctatgaacgttattgcaatattgaat

SEQ ID NO: 9 - DNA, 20 bp, Artificial Sequence
  Primer cadA-R2
agctgtttcctgtgtgaaat

SEQ ID NO: 10 - DNA, 39 bp, Artificial Sequence
  Primer K320A-F
accgacttcatcaaggcaacactggatgtgaaatccatc

SEQ ID NO: 11 - DNA, 39 bp, Artificial Sequence
  Primer K320A-R
gatttcacatccagtgttgccttgatgaagtcggtgttg

SEQ ID NO: 12 - DNA, 39 bp, Artificial Sequence
  Primer K320C-F
accgacttcatcaagtgcacactggatgtgaaatccatc

SEQ ID NO: 13 - DNA, 39 bp, Artificial Sequence
  Primer K320C-R
gatttcacatccagtgtgcacttgatgaagtcggtgttg

SEQ ID NO: 14 - DNA, 39 bp, Artificial Sequence
  Primer K320D-F
accgacttcatcaaggacacactggatgtgaaatccatc

SEQ ID NO: 15 - DNA, 39 bp, Artificial Sequence
  Primer K320D-R
gatttcacatccagtgtgtccttgatgaagtcggtgttg

SEQ ID NO: 16 - DNA, 39 bp, Artificial Sequence
  Primer K320E-F
accgacttcatcaaggaaacactggatgtgaaatccatc

SEQ ID NO: 17 - DNA, 39 bp, Artificial Sequence
  Primer K320E-R
gatttcacatccagtgtttccttgatgaagtcggtgttg

SEQ ID NO: 18 - DNA, 39 bp, Artificial Sequence
  Primer K320F-F
accgacttcatcaagttcacactggatgtgaaatccatc

SEQ ID NO: 19 - DNA, 39 bp, Artificial Sequence
  Primer K320F-R
gatttcacatccagtgtgaacttgatgaagtcggtgttg

SEQ ID NO: 20 - DNA, 39 bp, Artificial Sequence
  Primer K320G-F
accgacttcatcaagggaacactggatgtgaaatccatc

SEQ ID NO: 21 - DNA, 39 bp, Artificial Sequence
  Primer K320G-R
gatttcacatccagtgttcccttgatgaagtcggtgttg

SEQ ID NO: 22 - DNA, 39 bp, Artificial Sequence
  Primer K320H-F
accgacttcatcaagcatacactggatgtgaaatccatc

SEQ ID NO: 23 - DNA, 39 bp, Artificial Sequence
  Primer K320H-R
gatttcacatccagtgtatgcttgatgaagtcggtgttg

SEQ ID NO: 24 - DNA, 39 bp, Artificial Sequence
  Primer K320I-F
accgacttcatcaagatcacactggatgtgaaatccatc

SEQ ID NO: 25 - DNA, 39 bp, Artificial Sequence
  Primer K320I-R
gatttcacatccagtgtgatcttgatgaagtcggtgttg

SEQ ID NO: 26 - DNA, 39 bp, Artificial Sequence
  Primer K320L-F
accgacttcatcaagctgacactggatgtgaaatccatc

SEQ ID NO: 27 - DNA, 39 bp, Artificial Sequence
  Primer K320L-R
gatttcacatccagtgtcagcttgatgaagtcggtgttg

SEQ ID NO: 28 - DNA, 39 bp, Artificial Sequence
  Primer K320M-F
accgacttcatcaagatgacactggatgtgaaatccatc

SEQ ID NO: 29 - DNA, 39 bp, Artificial Sequence
  Primer K320M-R
gatttcacatccagtgtcatcttgatgaagtcggtgttg

SEQ ID NO: 30 - DNA, 39 bp, Artificial Sequence
  Primer K320N-F
accgacttcatcaagaacacactggatgtgaaatccatc

SEQ ID NO: 31 - DNA, 39 bp, Artificial Sequence
  Primer K320N-R
gatttcacatccagtgtgttcttgatgaagtcggtgttg

SEQ ID NO: 32 - DNA, 39 bp, Artificial Sequence
  Primer K320P-F
accgacttcatcaagccaacactggatgtgaaatccatc

SEQ ID NO: 33 - DNA, 39 bp, Artificial Sequence
  Primer K320P-R
gatttcacatccagtgttggcttgatgaagtcggtgttg

SEQ ID NO: 34 - DNA, 39 bp, Artificial Sequence
  Primer K320Q-F
accgacttcatcaagcaaacactggatgtgaaatccatc

SEQ ID NO: 35 - DNA, 39 bp, Artificial Sequence
  Primer K320Q-R
gatttcacatccagtgtttgcttgatgaagtcggtgttg

SEQ ID NO: 36 - DNA, 39 bp, Artificial Sequence
  Primer K320R-F
accgacttcatcaagcgtacactggatgtgaaatccatc

SEQ ID NO: 37 - DNA, 39 bp, Artificial Sequence
  Primer K320R-R
gatttcacatccagtgtacgcttgatgaagtcggtgttg

SEQ ID NO: 38 - DNA, 39 bp, Artificial Sequence
  Primer K320S-F
accgacttcatcaagtcaacactggatgtgaaatccatc

SEQ ID NO: 39 - DNA, 39 bp, Artificial Sequence
  Primer K320S-R
gatttcacatccagtgttgacttgatgaagtcggtgttg

SEQ ID NO: 40 - DNA, 39 bp, Artificial Sequence
  Primer K320T-F
accgacttcatcaagacaacactggatgtgaaatccatc

SEQ ID NO: 41 - DNA, 39 bp, Artificial Sequence
  Primer K320T-R
gatttcacatccagtgttgtcttgatgaagtcggtgttg

SEQ ID NO: 42 - DNA, 39 bp, Artificial Sequence
  Primer K320V-F
accgacttcatcaaggtaacactggatgtgaaatccatc

SEQ ID NO: 43 - DNA, 39 bp, Artificial Sequence
  Primer K320V-R
gatttcacatccagtgttaccttgatgaagtcggtgttg

SEQ ID NO: 44 - DNA, 39 bp, Artificial Sequence
  Primer K320W-F
accgacttcatcaagtggacactggatgtgaaatccatc

SEQ ID NO: 45 - DNA, 39 bp, Artificial Sequence
  Primer K320W-R
gatttcacatccagtgtccacttgatgaagtcggtgttg

SEQ ID NO: 46 - DNA, 39 bp, Artificial Sequence
  Primer K320Y-F
accgacttcatcaagtacacactggatgtgaaatccatc

SEQ ID NO: 47 - DNA, 39 bp, Artificial Sequence
  Primer K320Y-R
gatttcacatccagtgtgtacttgatgaagtcggtgttg

SEQ ID NO: 48 - protein, 714 aa, SALMONELLA ENTERICA; identical to SEQ ID NO: 5

SEQ ID NO: 49 - protein, 715 aa, ESCHERICHIA; identical to SEQ ID NO: 2

SEQ ID NO: 50 - protein, 715 aa, KLEBSIELLA; identical to SEQ ID NO: 3

SEQ ID NO: 51 - protein, 715 aa, ENTEROBACTERIAECEAE; identical to SEQ ID NO: 4